European Patent Specification EP 3 999 637 B1, published April 2, 2025. Title: INTESTINAL ALKALINE PHOSPHATASE-BASED TREATMENTS OF METABOLIC DISORDERS. Applicant: Synthetic Biologics, Inc. The sequence listing filed with the application follows.

SEQUENCE LISTING (11 sequences)

SEQ ID NO: 1 - protein, 528 aa, Artificial Sequence
  Synthetic polymer.
MQGPWVLLLLGLRLQLSLGVIPAEEENPAFWNRQAAEALDAAKKLQPIQKVAKNLILFLGDGLGVPTVTATRILKGQKNGKLGPETPLAMDRFPYLALSKTYNVDRQVPDSAATATAYLCGVKANFQTIGLSAAARFNQCNTTRGNEVISVMNRAKQAGKSVGVVTTTRVQHASPAGTYAHTVNRNWYSDADMPASARQEGCQDIATQLISNMDIDVILGGGRKYMFPMGTPDPEYPADASQNGIRLDGKNLVQEWLAKHQGAWYVWNRTELMQASLDQSVTHLMGLFEPGDTKYEIHRDPTLDPSLMEMTEAALRLLSRNPRGFYLFVEGGRIDHGHHEGVAYQALTEAVMFDDAIERAGQLTSEEDTLTLVTADHSHVFSFGGYTLRGSSIFGLAPSKAQDSKAYTSILYGNGPGYVFNSGVRPDVNESESGSPDYQQQAAVPLSSETHGGEDVAVFARGPQAHLVHGVQEQSFVAHVMAFAACLEPYTACDLAPPACTTDAAHPVAASLPLLAGTLLLLGASAAP

SEQ ID NO: 2 - protein, 533 aa, Artificial Sequence
  Synthetic polymer.
MQGACVLLLLGLHLQLSLGLIPAEEENPAFWNRQAAQALDVAKKLQPIQTAAKNVILFLGDGMGVPTVTATRILKGQMNGKLGPETPLAMDQFPYVALSKTYNVDRQVPDSAGTATAYLCGVKGNYRTIGVSAAARYNQCNTTRGNEVTSVINRAKKAGKAVGVVTTTRVQHASPAGAYAHTVNRNWYSDADLPADAQKNGCQDIAAQLVYNMDIDVILGGGRMYMFPEGTPDPEYPDDASVNGVRKDKQNLVQEWQAKHQGAQYVWNRTALLQAADDSSVTHLMGLFEPADMKYNVQQDHTKDPTLAEMTEAALQVLSRNPRGFYLFVEGGRIDHGHHDGKAYMALTEAIMFDNAIAKANELTSELDTLILVTADHSHVFSFGGYTLRGTSIFGLAPGKALDSKSYTSILYGNGPGYALGGGSRPDVNGSTSEEPSYRQQAAVPLASETHGGEDVAVFARGPQAHLVHGVQEETFVAHIMAFAGCVEPYTDCNLPAPATATSIPDAAHLAASPPPLALLAGAMLLLLAPTLY

SEQ ID NO: 3 - protein, 503 aa, Artificial Sequence
  Synthetic polymer.
MQGPWVLLLLGLRLQLSLGVIPAEEENPAFWNRQAAEALDAAKKLQPIQKVAKNLILFLGDGLGVPTVTATRILKGQKNGKLGPETPLAMDRFPYLALSKTYNVDRQVPDSAATATAYLCGVKANFQTIGLSAAARFNQCNTTRGNEVISVMNRAKQAGKSVGVVTTTRVQHASPAGTYAHTVNRNWYSDADMPASARQEGCQDIATQLISNMDIDVILGGGRKYMFPMGTPDPEYPADASQNGIRLDGKNLVQEWLAKHQGAWYVWNRTELMQASLDQSVTHLMGLFEPGDTKYEIHRDPTLDPSLMEMTEAALRLLSRNPRGFYLFVEGGRIDHGHHEGVAYQALTEAVMFDDAIERAGQLTSEEDTLTLVTADHSHVFSFGGYTLRGSSIFGLAPSKAQDSKAYTSILYGNGPGYVFNSGVRPDVNESESGSPDYQQQAAVPLSSETHGGEDVAVFARGPQAHLVHGVQEQSFVAHVMAFAACLEPYTACDLAPPAGTTD

SEQ ID NO: 4 - protein, 506 aa, Artificial Sequence
  Synthetic polymer.
MQGACVLLLLGLHLQLSLGLIPAEEENPAFWNRQAAQALDVAKKLQPIQTAAKNVILFLGDGMGVPTVTATRILKGQMNGKLGPETPLAMDQFPYVALSKTYNVDRQVPDSAGTATAYLCGVKGNYRTIGVSAAARYNQCNTTRGNEVTSVINRAKKAGKAVGVVTTTRVQHASPAGAYAHTVNRNWYSDADLPADAQKNGCQDIAAQLVYNMDIDVILGGGRMYMFPEGTPDPEYPDDASVNGVRKDKQNLVQEWQAKHQGAQYVWNRTALLQAADDSSVTHLMGLFEPADMKYNVQQDHTKDPTLAEMTEAALQVLSRNPRGFYLFVEGGRIDHGHHDGKAYMALTEAIMFDNAIAKANELTSELDTLILVTADHSHVFSFGGYTLRGTSIFGLAPGKALDSKSYTSILYGNGPGYALGGGSRPDVNGSTSEEPSYRQQAAVPLASETHGGEDVAVFARGPQAHLVHGVQEETFVAHIMAFAGCVEPYTDCNLPAPATATSIPD

SEQ ID NO: 5 - protein, 754 aa, Artificial Sequence
  Synthetic polymer.
MQGACVLLLLGLHLQLSLGLIPAEEENPAFWNRQAAQALDVAKKLQPIQTAAKNVILFLGDGMGVPTVTATRILKGQMNGKLGPETPLAMDQFPYVALSKTYNVDRQVPDSAGTATAYLCGVKGNYRTIGVSAAARYNQCNTTRGNEVTSVINRAKKAGKAVGVVTTTRVQHASPAGAYAHTVNRNWYSDADLPADAQKNGCQDIAAQLVYNMDIDVILGGGRMYMFPEGTPDPEYPDDASVNGVRKDKQNLVQEWQAKHQGAQYVWNRTALLQAADDSSVTHLMGLFEPADMKYNVQQDHTKDPTLAEMTEAALQVLSRNPRGFYLFVEGGRIDHGHHDGKAYMALTEAIMFDNAIAKANELTSELDTLILVTADHSHVFSFGGYTLRGTSIFGLAPGKALDSKSYTSILYGNGPGYALGGGSRPDVNGSTSEEPSYRQQAAVPLASETHGGEDVAVFARGPQAHLVHGVQEETFVAHIMAFAGCVEPYTDCNLPAPATATSIPDGGSGGSGGGGSGGGGSEPKSCDKTHTCPPCPAPELLGGPSVFLFPPKPKDTLMISRTPEVTCVVVDVSHEDPQVKFNWYVDGVQVHNAKTKPREQQYNSTYRVVSVLTVLHQNWLDGKEYKCKVSNKALPAPIEKTISKAKGQPREPQVYTLPPSREEMTKNQVSLTCLVKGFYPSDIAVEWESNGQPENNYKTTPPVLDSDGSFFLYSKLTVDKSRWQQGNVFSCSVMHEALHNHYTQKSLSLSPGK

SEQ ID NO: 6 - protein, 534 aa, Artificial Sequence
  Synthetic polymer.
MQWACVLLLLGLWLQLSLTFIPAEEEDPAFWNRQAAQALDVAKKLQPIQTAAKNVILFLGDGMGVPTVTATRILKGQMNGKLGPETPLAMDQFPYVALSKTYNVDRQVPDSAGTATAYLCGVKGNYKTIGVSAAARYNQCNTTSGNEVTSVMNRAKKAGKSVGVVTTSRVQHASPAGAYAHTVNRNWYSDADLPADAQTYGCQDIATQLVNNMDIDVILGGGRMYMFPEGTPDPEYPYDVNQTGVRKDKRNLVQEWQAKHQGAQYVWNRTELLQAANDPSVTHLMGLFEPADMKYNVQQDPTKDPTLEEMTEAALQVLSRNPQGFYLFVEGGRIDHGHHEGKAYMALTDTVMFDNAIAKANELTSELDTLILATADHSHVFSFGGYTLRGTSIFGLAPSKASDNKSYTSILYGNGPGYVLGGGLRPDVNDSISEDPSYRQQAAVPLSSESHGGEDVAVFARGPQAHLVHGVQEETFVAHVMAFAGCVEPYTDCNLAPPAGTTDAAHPIEGRSVVPALLPLRAGTLLLLETATAP

SEQ ID NO: 7 - DNA, 1669 bp, Artificial Sequence
  Synthetic polymer.
atgcaggggccctgggtgctgctgctgctgggcctgaggctacagctctccctgggcgtcatcccaggtaatgaggctccccaagctgttccacacacagggcaccccctcagccaggctgacctgatctctactctccccctggccagctgaggaggagaacccggccttctggaaccgccaggcagctgaggccctggatgctgccaagaagctgcagcccatccagaaggtcgccaagaacctcatcctcttcctgggcgatgggttgggggtgcccacggtgacagccaccaggatcctaaaggggcagaagaatggcaaactggggcctgagacgcccctggccatggaccgcttcccatacctggctctgtccaagacatacaatgtggacagacaggtgccagacagcgcagccacagccacggcctacctgtgcggggtcaaggccaacttccagaccatcggcttgagtgcagccgcccgctttaaccagtgcaacacgacacgcggcaatgaggtcatctccgtgatgaaccgggccaagcaagcaggaaagtcagtaggagtggtgaccaccacacgggtgcagcacgcctcgccagccggcacctacgcacacacagtgaaccgcaactggtactcagatgctgacatgcctgcctcagcccgccaggaggggtgccaggacatcgccactcagctcatctccaacatggacattgacgtgatccttggcggaggccgcaagtacatgtttcccatggggaccccagaccctgagtacccagctgatgccagccagaatggaatcaggctggacgggaagaacctggtgcaggaatggctggcaaagcaccagggtgcctggtatgtgtggaaccgcactgagctcatgcaggcgtccctggaccagtctgtgacccatctcatgggcctctttgagcccggagacacgaaatatgagatccaccgagaccccacactggacccctccctgatggagatgacagaggctgccctgcgcctgctgagcaggaacccccgcggcttctacctctttgtggagggcggccgcatcgaccatggtcatcatgagggtgtggcttaccaggcactcactgaggcggtcatgttcgacgacgccattgagagggcgggccagctcaccagcgaggaggacacgctgaccctcgtcaccgctgaccactcccatgtcttctcctttggtggctacaccttgcgagggagctccatcttcgggttggcccccagcaaggctcaggacagcaaagcctacacgtccatcctgtacggcaatggcccgggctacgtgttcaactcaggcgtgcgaccagacgtgaatgagagcgagagcgggagccccgattaccagcagcaggcggcggtgcccctgtcgtccgagacccacggaggcgaagacgtggcggtgtttgcgcgcggcccgcaggcgcacctggtgcatggtgtgcaggagcagagcttcgtagcgcatgtcatggccttcgctgcctgtctggagccctacacggcctgcgacctggcgcctcccgcctgcaccaccgacgccgcgcacccagttgccgcgtcgctgccactgctggccgggaccctgctgctgctgggggcgtccgctgctccctga

SEQ ID NO: 8 - DNA, 1671 bp, Artificial Sequence
  Synthetic polymer.
atgcaggggccctgggtgctgctgctgctgggcctgaggctacagctctccctgggcgtcatcccagctgaggaggagaacccggccttctggaaccgccaggcagctgaggccctggatgctgccaagaagctgcagcccatccagaaggtcgccaagaacctcatcctcttcctgggcgatgggttgggggtgcccacggtgacagccaccaggatcctaaaggggcagaagaatggcaaactggggcctgagacgcccctggccatggaccgcttcccatacctggctctgtccaagacatacaatgtggacagacaggtgccagacagcgcagccacagccacggcctacctgtgcggggtcaaggccaacttccagaccatcggcttgagtgcagccgcccgctttaaccagtgcaacacgacacgcggcaatgaggtcatctccgtgatgaaccgggccaagcaagcaggaaagtcagtaggagtggtgaccaccacacgggtgcagcacgcctcgccagccggcacctacgcacacacagtgaaccgcaactggtactcagatgctgacatgcctgcctcagcccgccaggaggggtgccaggacatcgccactcagctcatctccaacatggacattgacgtgatccttggcggaggccgcaagtacatgtttcccatggggaccccagaccctgagtacccagctgatgccagccagaatggaatcaggctggacgggaagaacctggtgcaggaatggctggcaaagcaccagggtgcctggtatgtgtggaaccgcactgagctcatgcaggcgtccctggaccagtctgtgacccatctcatgggcctctttgagcccggagacacgaaatatgagatccaccgagaccccacactggacccctccctgatggagatgacagaggctgccctgcgcctgctgagcaggaacccccgcggcttctacctctttgtggagggcggccgcatcgaccatggtcatcatgagggtgtggcttaccaggcactcactgaggcggtcatgttcgacgacgccattgagagggcgggccagctcaccagcgaggaggacacgctgaccctcgtcaccgctgaccactcccatgtcttctcctttggtggctacaccttgcgagggagctccatcttcgggttggcccccagcaaggctcaggacagcaaagcctacacgtccatcctgtacggcaatggcccgggctacgtgttcaactcaggcgtgcgaccagacgtgaatgagagcgagagcgggagccccgattaccagcagcaggcggcggtgcccctgtcgtccgagacccacggaggcgaagacgtggcggtgtttgcgcgcggcccgcaggcgcacctggtgcatggtgtgcaggagcagagcttcgtagcgcatgtcatggccttcgctgcctgtctggagccctacacggcctgcgacctggcgcctcccgcctgcaccaccgacgccgcgcacccagttgccgcgtcgctgccactgctggccgggaccctgctgctgctgggggcgtccgctgctccctgatttactaaaaccttgaaataaaattgtaaaacatcagtttgaaggcctgactctcagggtagttcttttttaattctgggtttt

SEQ ID NO: 9 - DNA, 1259 bp, Artificial Sequence
  Synthetic polymer.
aaaaaacaagacaaagctgagatcagaaatgtcattgtgatgataggcgacggcatggggacgccttacataagagcctaccgttccatgaaaaataacggtgacacaccgaataacccgaagttaacagaatttgaccggaacctgacaggcatgatgatgacgcatccggatgaccctgactataatattacagattcagcagcagccggaacagcattagcgacaggcgttaagacatataacaatgcaattggcgtcgataaaaacggaaaaaaagtgaaatctgtacttgaagaggccaaacagcaaggcaagtcaacagggcttgtcgccacgtctgaaattaaccacgccactccagccgcatatggcgcccacaatgaatcacggaaaaacatggaccaaatcgccaacagctatatggatgacaagataaaaggcaaacataaaatagacgtgctgctcggcggcggaaaatcttattttaaccgcaagaacagaaacttgacaaaggaattcaaacaagccggctacagctatgtgacaactaaacaagcattgaaaaaaaataaagatcagcaggtgctcgggcttttcgcagatggagggcttgctaaagcgctcgaccgtgacagtaaaacaccgtctctcaaagacatgacggtttcagcaattgatcgcctgaaccaaaataaaaaaggatttttcttgatggtcgaagggagccagattgactgggcggcccatgacaatgatacagtaggagccatgagcgaggttaaagattttgaacaggcctataaagccgcgattgaatttgcgaaaaaagacaaacatacacttgtgattgcaactgctgaccatacaaccggcggctttaccattggcgcaaacggggaaaagaattggcacgcagaaccgattctctccgctaagaaaacacctgaattcatggccaaaaaaatcaggaaggcaagccggttaaagatgtgctcgcccgctatgccaatctgaaagtcacatctgaagaaatcaaaagcgttgaagcagctgcacaggctgacaaaagcaaaggggcctccaaagccatcatcaagatttttaatacccgctccaacagcggatggacgagtaccgatcataccggcgaagaagtaccggtatacgcgtacggccccggaaaagaaaaattccgcggattgattaacaatacggaccaggcaaacatcatatttaagattttaaaaactggaaaa

SEQ ID NO: 10 - protein, 420 aa, Artificial Sequence
  Synthetic polymer.
KKQDKAEIRNVIVMIGDGMGTPYIRAYRSMKNNGDTPNNPKLTEFDRNLTGMMMTHPDDPDYNITDSAAAGTALATGVKTYNNAIGVDKNGKKVKSVLEEAKQQGKSTGLVATSEINHATPAAYGAHNESRKNMDQIANSYMDDKIKGKHKIDVLLGGGKSYFNRKNRNLTKEFKQAGYSYVTTKQALKKNKDQQVLGLFADGGLAKALDRDSKTPSLKDMTVSAIDRLNQNKKGFFLMVEGSQIDWAAHDNDTVGAMSEVKDFEQAYKAAIEFAKKDKHTLVIATADHTTGGFTIGANGEKNWHAEPILSAKKTPEFMAKKISEGKPVKDVLARYANLKVTSEEIKSVEAAAQADKSKGASKAIIKIFNTRSNSGWTSTDHTGEEVPVYAYGPGKEKFRGLINNTDQANIIFKILKTGK

SEQ ID NO: 11 - protein, 487 aa, Artificial Sequence
  Synthetic polymer.
LIPAEEENPAFWNRQAAQALDVAKKLQPIQTAAKNVILFLGDGMGVPTVTATRILKGQMNGKLGPETPLAMDQFPYVALSKTYNVDRQVPDSAGTATAYLCGVKGNYRTIGVSAAARYNQCNTTRGNEVTSVINRAKKAGKAVGVVTTTRVQHASPAGAYAHTVNRNWYSDADLPADAQKNGCQDIAAQLVYNMDIDVILGGGRMYMFPEGTPDPEYPDDASVNGVRKDKQNLVQEWQAKHQGAQYVWNRTALLQAADDSSVTHLMGLFEPADMKYNVQQDHTKDPTLAEMTEAALQVLSRNPRGFYLFVEGGRIDHGHHDGKAYMALTEAIMFDNAIAKANELTSELDTLILVTADHSHVFSFGGYTLRGTSIFGLAPGKALDSKSYTSILYGNGPGYALGGGSRPDVNGSTSEEPSYRQQAAVPLASETHGGEDVAVFARGPQAHLVHGVQEETFVAHIMAFAGCVEPYTDCNLPAPATATSIPD